European Patent Specification EP 3 896 162 B1, published March 5, 2025. Title: ARTIFICIALLY ENGINEERED SC FUNCTION CONTROL SYSTEM. Applicant: TOOLGEN INCORPORATED. Application pct/kr2017/010897. The sequence listing filed with the application follows.

SEQUENCE LISTING (234 sequences)

SEQ ID NO: 1 - DNA, 20 bp, Homo sapiens
cgatgatactcagcaacagg

SEQ ID NO: 2 - DNA, 20 bp, Homo sapiens
ggacgatgatactcagcaac

SEQ ID NO: 3 - DNA, 20 bp, Homo sapiens
atggacacgcaactgatctc

SEQ ID NO: 4 - DNA, 20 bp, Homo sapiens
gatgatcgacaggatcatgg

SEQ ID NO: 5 - DNA, 20 bp, Homo sapiens
gaagatgatcgacaggatca

SEQ ID NO: 6 - DNA, 20 bp, Homo sapiens
aactcttcaccctcaccaag

SEQ ID NO: 7 - DNA, 20 bp, Homo sapiens
aaaacctgccccccttggtg

SEQ ID NO: 8 - DNA, 20 bp, Homo sapiens
ggaatcttccaaattcttgc

SEQ ID NO: 9 - DNA, 22 bp, Homo sapiens
gatcgtggagacgaacagcagc

SEQ ID NO: 10 - DNA, 22 bp, Homo sapiens
gctgacgatcgtggagacgaac

SEQ ID NO: 11 - DNA, 22 bp, Homo sapiens
cgcaactgatctctggcagaac

SEQ ID NO: 12 - DNA, 22 bp, Homo sapiens
gtgcgtgatgagtgctgcggcc

SEQ ID NO: 13 - DNA, 22 bp, Homo sapiens
gtgtagatggccgcagcactca

SEQ ID NO: 14 - DNA, 20 bp, Homo sapiens
ggaccagcccctgaataaac

SEQ ID NO: 15 - DNA, 20 bp, Homo sapiens
ggcgtctttccagtttattc

SEQ ID NO: 16 - DNA, 20 bp, Homo sapiens
gcgtctttccagtttattca

SEQ ID NO: 17 - DNA, 20 bp, Homo sapiens
cgtctttccagtttattcag

SEQ ID NO: 18 - DNA, 20 bp, Homo sapiens
ttcaggggctggtccaatgc

SEQ ID NO: 19 - DNA, 20 bp, Homo sapiens
tcaggggctggtccaatgct

SEQ ID NO: 20 - DNA, 20 bp, Homo sapiens
accatgacatatcccagcat

SEQ ID NO: 21 - DNA, 20 bp, Homo sapiens
tttccagtttattcaggggc

SEQ ID NO: 22 - DNA, 20 bp, Homo sapiens
cagttacagggagcaccacc

SEQ ID NO: 23 - DNA, 20 bp, Homo sapiens
ctggtctggcttcagttaca

SEQ ID NO: 24 - DNA, 20 bp, Homo sapiens
cctggtctggcttcagttac

SEQ ID NO: 25 - DNA, 20 bp, Homo sapiens
aactggaaagacgcctggtc

SEQ ID NO: 26 - DNA, 20 bp, Homo sapiens
gaataaactggaaagacgcc

SEQ ID NO: 27 - DNA, 20 bp, Homo sapiens
tccaatgctgggatatgtca

SEQ ID NO: 28 - DNA, 20 bp, Homo sapiens
aatgctgggatatgtcatgg

SEQ ID NO: 29 - DNA, 20 bp, Homo sapiens
atagaggctgagaacctctc

SEQ ID NO: 30 - DNA, 22 bp, Homo sapiens
gccctctgaatctccagtcaat

SEQ ID NO: 31 - DNA, 22 bp, Homo sapiens
aatctccagtcaattccaacac

SEQ ID NO: 32 - DNA, 22 bp, Homo sapiens
aattaggcaattcttgtaaagc

SEQ ID NO: 33 - DNA, 22 bp, Homo sapiens
ttaggcaattcttgtaaagcat

SEQ ID NO: 34 - DNA, 22 bp, Homo sapiens
aaagcataggcacacatcaccc

SEQ ID NO: 35 - DNA, 22 bp, Homo sapiens
gcctggtctggcttcagttaca

SEQ ID NO: 36 - DNA, 22 bp, Homo sapiens
gtgtccaactttgtttgctttc

SEQ ID NO: 37 - DNA, 22 bp, Homo sapiens
gtattctggaaagcaaacaaag

SEQ ID NO: 38 - DNA, 22 bp, Homo sapiens
cagtcttggcatcacaggcttc

SEQ ID NO: 39 - DNA, 22 bp, Homo sapiens
ggacctcttggctattacacag

SEQ ID NO: 40 - DNA, 22 bp, Homo sapiens
ggagccagtgggacctcttggc

SEQ ID NO: 41 - DNA, 20 bp, Homo sapiens
ttgggcatgtttgagctggt

SEQ ID NO: 42 - DNA, 20 bp, Homo sapiens
tttgggcatgtttgagctgg

SEQ ID NO: 43 - DNA, 20 bp, Homo sapiens
gagctggtgggcgaagcata

SEQ ID NO: 44 - DNA, 20 bp, Homo sapiens
agctggtgggcgaagcatat

SEQ ID NO: 45 - DNA, 20 bp, Homo sapiens
tgggcgaagcatatgggcaa

SEQ ID NO: 46 - DNA, 20 bp, Homo sapiens
ggcctccatcctaaacaatg

SEQ ID NO: 47 - DNA, 20 bp, Homo sapiens
gggttgggaggtttgggcgt

SEQ ID NO: 48 - DNA, 20 bp, Homo sapiens
aggtttgggcgtgggagtcc

SEQ ID NO: 49 - DNA, 19 bp, Homo sapiens
ttcagagactcagctattt

SEQ ID NO: 50 - DNA, 19 bp, Homo sapiens
ggccacattgtttaggatg

SEQ ID NO: 51 - DNA, 19 bp, Homo sapiens
ggctttgggcatgtttgag

SEQ ID NO: 52 - DNA, 19 bp, Homo sapiens
aacatgcccaaagcccagc

SEQ ID NO: 53 - DNA, 19 bp, Homo sapiens
acatgcccaaagcccagcg

SEQ ID NO: 54 - DNA, 23 bp, Homo sapiens
ttaaatcacagaggcaaagagtt

SEQ ID NO: 55 - DNA, 22 bp, Homo sapiens
ttgcatagtgctagactgtttt

SEQ ID NO: 56 - DNA, 22 bp, Homo sapiens
gggtcatgtgttttgaaaacag

SEQ ID NO: 57 - DNA, 22 bp, Homo sapiens
cccaaacctcccaacccacaac

SEQ ID NO: 58 - DNA, 22 bp, Homo sapiens
actcagctatttctggaatgac

SEQ ID NO: 59 - DNA, 22 bp, Homo sapiens
tcatcgcctttgtgagctccat

SEQ ID NO: 60 - DNA, 22 bp, Homo sapiens
cagacacaggctttgctctagc

SEQ ID NO: 61 - DNA, 22 bp, Homo sapiens
caaagcctgtgtctggccacta

SEQ ID NO: 62 - DNA, 22 bp, Homo sapiens
agcagtttgtgcccactagtgg

SEQ ID NO: 63 - DNA, 22 bp, Homo sapiens
atgtcaaggtattccagctaac

SEQ ID NO: 64 - DNA, 22 bp, Homo sapiens
gaataactgtatcaaagttagc

SEQ ID NO: 65 - DNA, 22 bp, Homo sapiens
ttcctaattaagaggctttgtg

SEQ ID NO: 66 - DNA, 22 bp, Homo sapiens
gagctagtttgtcagggtctag

SEQ ID NO: 67 - DNA, 20 bp, Artificial Sequence
  primer
cacagggcagtcagagaccc

SEQ ID NO: 68 - DNA, 20 bp, Artificial Sequence
  primer
gcaaacaaagttggacactg

SEQ ID NO: 69 - DNA, 24 bp, Artificial Sequence
  primer
agactcccgcccatcttctagaaa

SEQ ID NO: 70 - DNA, 24 bp, Artificial Sequence
  primer
aagtcgctctgagttgttatcagt

SEQ ID NO: 71 - DNA, 19 bp, Artificial Sequence
  primer
cagtgaaacgcaccagacg

SEQ ID NO: 72 - DNA, 20 bp, Artificial Sequence
  primer
aatctgcctaacaggaggtg

SEQ ID NO: 73 - DNA, 24 bp, Artificial Sequence
  primer
gagggaatggggaccaaaggcatt

SEQ ID NO: 74 - DNA, 24 bp, Artificial Sequence
  primer
tcatgtggggtgatgttcaggaag

SEQ ID NO: 75 - DNA, 23 bp, Artificial Sequence
  primer
agagcagctgacctgaggtccaa

SEQ ID NO: 76 - DNA, 24 bp, Artificial Sequence
  primer
cccaagggtagagtgcaagtaaac

SEQ ID NO: 77 - DNA, 24 bp, Artificial Sequence
  primer
gcatcctagctcatttggtctgct

SEQ ID NO: 78 - DNA, 24 bp, Artificial Sequence
  primer
gagaggattcctcatgaatgggat

SEQ ID NO: 79 - DNA, 24 bp, Artificial Sequence
  primer
accaaacactacacttggttactg

SEQ ID NO: 80 - DNA, 24 bp, Artificial Sequence
  primer
ctcccactagcaattttaaagtct

SEQ ID NO: 81 - DNA, 24 bp, Artificial Sequence
  primer
gaatgttcagcacaggtttccttg

SEQ ID NO: 82 - DNA, 24 bp, Artificial Sequence
  primer
ggtcaaaaggagctccatatttga

SEQ ID NO: 83 - DNA, 24 bp, Artificial Sequence
  primer
caggacacccatggccaaatccag

SEQ ID NO: 84 - DNA, 24 bp, Artificial Sequence
  primer
cagagcctcctgcagggatgtcaa

SEQ ID NO: 85 - DNA, 24 bp, Artificial Sequence
  primer
gcctgccaaggtgactctcatcta

SEQ ID NO: 86 - DNA, 24 bp, Artificial Sequence
  primer
tgcccaggctgatcttgaactcct

SEQ ID NO: 87 - DNA, 24 bp, Artificial Sequence
  primer
cccagagttaagaggttctttcct

SEQ ID NO: 88 - DNA, 24 bp, Artificial Sequence
  primer
gaagctactccagtgcaactagct

SEQ ID NO: 89 - DNA, 23 bp, Artificial Sequence
  primer
acgcagtctgttctgtgcagtgt

SEQ ID NO: 90 - DNA, 24 bp, Artificial Sequence
  primer
aggccttcccaaggaagaccctga

SEQ ID NO: 91 - DNA, 24 bp, Artificial Sequence
  primer
gctgatcactggccaaatccagct

SEQ ID NO: 92 - DNA, 24 bp, Artificial Sequence
  primer
gggaaacaatgggatcaagctgca

SEQ ID NO: 93 - DNA, 24 bp, Artificial Sequence
  primer
gcccctttgtaagttgaggagcat

SEQ ID NO: 94 - DNA, 24 bp, Artificial Sequence
  primer
ccctctacctctctcaatgggctt

SEQ ID NO: 95 - DNA, 24 bp, Artificial Sequence
  primer
cagacaagcaaatgctgagagatt

SEQ ID NO: 96 - DNA, 24 bp, Artificial Sequence
  primer
cctgtcattatgatgttcgctagt

SEQ ID NO: 97 - DNA, 24 bp, Artificial Sequence
  primer
ccagagttggcctcctacagagat

SEQ ID NO: 98 - DNA, 24 bp, Artificial Sequence
  primer
gtggatgccccactactgttcatt

SEQ ID NO: 99 - DNA, 24 bp, Artificial Sequence
  primer
tacccaatttgccagtctgtgtct

SEQ ID NO: 100 - DNA, 23 bp, Artificial Sequence
  primer
accaccaggcctgccctacaaga

SEQ ID NO: 101 - DNA, 24 bp, Artificial Sequence
  primer
tgtgaatttgatcctggcattatg

SEQ ID NO: 102 - DNA, 24 bp, Artificial Sequence
  primer
tacagacaagcagatgctgagaga

SEQ ID NO: 103 - DNA, 24 bp, Artificial Sequence
  primer
cagtcaacagagctctaacctcct

SEQ ID NO: 104 - DNA, 23 bp, Artificial Sequence
  primer
agcacctggttgcacatcaactt

SEQ ID NO: 105 - DNA, 24 bp, Artificial Sequence
  primer
catgtggtccctgaacgtgaatga

SEQ ID NO: 106 - DNA, 23 bp, Artificial Sequence
  primer
gtctgtcgcttgccctcttctct

SEQ ID NO: 107 - DNA, 24 bp, Artificial Sequence
  primer
atgcagggcctctagaccatttca

SEQ ID NO: 108 - DNA, 23 bp, Artificial Sequence
  primer
ctcagccctttgtgcactcacct

SEQ ID NO: 109 - DNA, 20 bp, Artificial Sequence
  primer
tgcacatcgcaaacatttcg

SEQ ID NO: 110 - DNA, 20 bp, Artificial Sequence
  primer
tgggtatcgcactgtgtcag

SEQ ID NO: 111 - DNA, 20 bp, Artificial Sequence
  primer
aggttcacatggcttgtggt

SEQ ID NO: 112 - DNA, 20 bp, Artificial Sequence
  primer
atatctgaaatgcccgcagg

SEQ ID NO: 113 - DNA, 20 bp, Artificial Sequence
  primer
tgcacatcgcaaacatttcg

SEQ ID NO: 114 - DNA, 20 bp, Artificial Sequence
  primer
tgggtatcgcactgtgtcag

SEQ ID NO: 115 - DNA, 20 bp, Artificial Sequence
  primer
tctttaaaggccttatctcc

SEQ ID NO: 116 - DNA, 20 bp, Artificial Sequence
  primer
ttctgcttgagaattcatcc

SEQ ID NO: 117 - DNA, 20 bp, Artificial Sequence
  primer
ctcctaatctttcacttagg

SEQ ID NO: 118 - DNA, 20 bp, Artificial Sequence
  primer
caaagcctggtataacatag

SEQ ID NO: 119 - DNA, 19 bp, Artificial Sequence
  primer
tcacttcgagcatctgtgg

SEQ ID NO: 120 - DNA, 19 bp, Artificial Sequence
  primer
ccaaatgacaggctgagct

SEQ ID NO: 121 - DNA, 20 bp, Artificial Sequence
  primer
agcaggaagtgaaggctaag

SEQ ID NO: 122 - DNA, 20 bp, Artificial Sequence
  primer
atgtaacgtggcaactctgg

SEQ ID NO: 123 - DNA, 20 bp, Artificial Sequence
  primer
gtgttgctctcgtcaattag

SEQ ID NO: 124 - DNA, 20 bp, Artificial Sequence
  primer
aggtgttgtacatggagaag

SEQ ID NO: 125 - DNA, 20 bp, Artificial Sequence
  primer
tgtgagccaccatacccagc

SEQ ID NO: 126 - DNA, 20 bp, Artificial Sequence
  primer
cctgcagtcctttgcggatc

SEQ ID NO: 127 - DNA, 20 bp, Artificial Sequence
  primer
tcgctgccagtataacatgc

SEQ ID NO: 128 - DNA, 20 bp, Artificial Sequence
  primer
aactccagtctctagactcg

SEQ ID NO: 129 - DNA, 20 bp, Artificial Sequence
  primer
aatagtttgacgttggagcc

SEQ ID NO: 130 - DNA, 20 bp, Artificial Sequence
  primer
actcccaacatgttctcctg

SEQ ID NO: 131 - DNA, 19 bp, Artificial Sequence
  primer
atcatcgctcacagagtcc

SEQ ID NO: 132 - DNA, 20 bp, Artificial Sequence
  primer
acgactgcaggatcttaatg

SEQ ID NO: 133 - DNA, 20 bp, Artificial Sequence
  primer
tggatggaggttgggaatcc

SEQ ID NO: 134 - DNA, 20 bp, Artificial Sequence
  primer
ttgaggcagcagcactctcc

SEQ ID NO: 135 - DNA, 19 bp, Artificial Sequence
  primer
agtctatcctagcagctcc

SEQ ID NO: 136 - DNA, 20 bp, Artificial Sequence
  primer
actgagaccagataatgcag

SEQ ID NO: 137 - DNA, 19 bp, Artificial Sequence
  primer
aagagatgcgagttgttcc

SEQ ID NO: 138 - DNA, 19 bp, Artificial Sequence
  primer
cctcttctactctgagtgg

SEQ ID NO: 139 - DNA, 20 bp, Artificial Sequence
  primer
acctggtttatcacaagcta

SEQ ID NO: 140 - DNA, 20 bp, Artificial Sequence
  primer
aacgtgaacagaaggatttc

SEQ ID NO: 141 - DNA, 20 bp, Artificial Sequence
  primer
atcactccatcagagtcagg

SEQ ID NO: 142 - DNA, 20 bp, Artificial Sequence
  primer
tggctccttctattctctcc

SEQ ID NO: 143 - DNA, 23 bp, Homo sapiens
tatggaattcccaagccccctgg

SEQ ID NO: 144 - DNA, 23 bp, Homo sapiens
ggaattccatatgagtcatctgg

SEQ ID NO: 145 - DNA, 23 bp, Homo sapiens
cacagcctacactttgattatgg

SEQ ID NO: 146 - DNA, 23 bp, Homo sapiens
tcaggagcattaagcatataggg

SEQ ID NO: 147 - DNA, 23 bp, Homo sapiens
gaccacggtccatgaattcctgg

SEQ ID NO: 148 - DNA, 23 bp, Homo sapiens
agtatttgcagctgaacaaaagg

SEQ ID NO: 149 - DNA, 23 bp, Homo sapiens
atggagtacagagagacataagg

SEQ ID NO: 150 - DNA, 23 bp, Homo sapiens
aaagaatcaatgcacagccatgg

SEQ ID NO: 151 - RNA, 12 nt, Artificial Sequence
  first complementary domain
guuuuagagcua

SEQ ID NO: 152 - RNA, 25 nt, Artificial Sequence
  first complementary domain
guuuuagucccuuuuuaaauuucuu

SEQ ID NO: 153 - RNA, 22 nt, Artificial Sequence
  firtst complementary domain
guuuuagagcuguguuguuucg

SEQ ID NO: 154 - RNA, 9 nt, Artificial Sequence
  first complementary domain
uuuguagau

SEQ ID NO: 155 - RNA, 14 nt, Artificial Sequence
  second complementary domain
uagcaaguuaaaau

SEQ ID NO: 156 - RNA, 24 nt, Artificial Sequence
  second complementary domain
cgaaacaacacagcgaguuaaaau

SEQ ID NO: 157 - RNA, 25 nt, Artificial Sequence
  second complementary domain
aagaaauuuaaaaagggacuaaaau

SEQ ID NO: 158 - RNA, 12 nt, Artificial Sequence
  proximal domain
aaggcuaguccg

SEQ ID NO: 159 - RNA, 11 nt, Artificial Sequence
  proximal domain
aaagaguuugc

SEQ ID NO: 160 - RNA, 11 nt, Artificial Sequence
  second complementary domain
aaauuucuacu

SEQ ID NO: 161 - RNA, 34 nt, Artificial Sequence
  tail domain
uuaucaacuugaaaaaguggcaccgagucggugc

SEQ ID NO: 162 - RNA, 38 nt, Artificial Sequence
  tail domain
gggacucugcgggguuacaauccccuaaaaccgcuuuu

SEQ ID NO: 163 - RNA, 38 nt, Artificial Sequence
  tail domain
uacucaacuugaaaagguggcaccgauucgguguuuuu

SEQ ID NO: 164 - RNA, 76 nt, Artificial Sequence
  sgRNA backbone
guuuuagagcuagaaauagcaaguuaaaauaaggcuaguccguuaucaacuugaaaaaguggcaccgagucggugc

SEQ ID NO: 165 - RNA, 13 nt, Artificial Sequence
  proximal domain
aaggcuuaguccg

SEQ ID NO: 166 - RNA, 77 nt, Artificial Sequence
  sgRNA backbone
guuuuagucccugaaaagggacuaaaauaaagaguuugcgggacucugcgggguuacaauccccuaaaaccgcuuuu

SEQ ID NO: 167 - protein, 16 aa, Artificial Sequence
  nuclear localization sequence
KRPAATKKAGQAKKKK

SEQ ID NO: 168 - protein, 11 aa, Artificial Sequence
  nuclear localization sequence
RQRRNELKRSP

SEQ ID NO: 169 - protein, 38 aa, Artificial Sequence
  nuclear localization sequence
NQSSNFGPMKGGNFGGRSSGPYGGGGQYFAKPRNQGGY

SEQ ID NO: 170 - protein, 42 aa, Artificial Sequence
  nuclear localization sequence
RMRIZFKNKGKDTAELRRRRVEVSVELRKAKKDEQILKRRNV

SEQ ID NO: 171 - protein, 12 aa, Artificial Sequence
  nuclear localization sequence
SALIKKKKKMAP

SEQ ID NO: 172 - protein, 10 aa, Artificial Sequence
  nuclear localization sequence
RKLKKKIKKL

SEQ ID NO: 173 - protein, 10 aa, Artificial Sequence
  nuclear localization sequence
REKKKFLKRR

SEQ ID NO: 174 - protein, 20 aa, Artificial Sequence
  nuclear localization sequence
KRKGDEVDGVDEVAKKKSKK

SEQ ID NO: 175 - protein, 17 aa, Artificial Sequence
  nuclear localization sequence
RKCLQAGMNLEARKTKK

SEQ ID NO: 176 - protein, 7 aa, Artificial Sequence
  NLS of SV40 virus large T-antigen
PKKKRKV

SEQ ID NO: 177 - protein, 9 aa, Artificial Sequence
  c-myc NLS
PAAKRVKLD

SEQ ID NO: 178 - protein, 8 aa, Artificial Sequence
  myoma T protein sequences
VSRKRPRP

SEQ ID NO: 179 - protein, 8 aa, Artificial Sequence
  myoma T protein sequences
PPKKARED

SEQ ID NO: 180 - protein, 8 aa, Artificial Sequence
  human p53 sequence
PQPKKKPL

SEQ ID NO: 181 - protein, 5 aa, Artificial Sequence
  influenza virus NS1 sequences
DRLRR

SEQ ID NO: 182 - protein, 7 aa, Artificial Sequence
  influenza virus NS1 sequences
PKQKKRK

SEQ ID NO: 183 - DNA, 89 bp, Artificial Sequence
  Wild type Egr2
ggcctccatcctaaacaatgtggcctttgcccatatgcttcgcccaccagctcaaacatgcccaaagcccaaagcccagcgtgggtctt

SEQ ID NO: 184 - DNA, 23 bp, Artificial Sequence
  Enh-Sp5
cctttgcccatatgcttcgccca

SEQ ID NO: 185 - DNA, 23 bp, Artificial Sequence
  Enh-Sp16
acatgcccaaagcccagcgtggg

SEQ ID NO: 186 - DNA, 29 bp, Artificial Sequence
  mutant Egr2 part 1
ggcctccatcctaaacaatgtggcctttg

SEQ ID NO: 187 - DNA, 10 bp, Artificial Sequence
  mutant Egr2 part 2
cgtgggtctt

SEQ ID NO: 188 - DNA, 89 bp, Artificial Sequence
  wild type TATA
ggtgctccctgtaactgaagccagaccaggcgtctttccagtttattcaggggctggtccaatgctgggatatgtcatggtggcctgag

SEQ ID NO: 189 - DNA, 23 bp, Artificial Sequence
  TATA-Sp12
ccagaccaggcgtctttccagtt

SEQ ID NO: 190 - DNA, 23 bp, Artificial Sequence
  TATA-Sp14
tccaatgctgggatatgtcatgg

SEQ ID NO: 191 - DNA, 26 bp, Artificial Sequence
  mutant TATA part 1
ggtgctccctgtaactgaagccagac

SEQ ID NO: 192 - DNA, 15 bp, Artificial Sequence
  mutant TATA part 2
tcatggtggcctgag

SEQ ID NO: 193 - DNA, 120 bp, Artificial Sequence
  promoter chain 1
cctggtggtgctccctgtaactgaagccagaccaggcgtctttccagtttattcaggggctggtccaatgctgggatatgtcatggtggcctgagaggttctcagcctctattatttaaa

SEQ ID NO: 194 - DNA, 120 bp, Artificial Sequence
  promoter part 2
ggaccaccacgagggacattgacttcggtctggtccgcagaaaggtcaaataagtccccgaccaggttacgaccctatacagtaccaccggactctccaagagtcggagataataaattt

SEQ ID NO: 195 - DNA, 90 bp, Artificial Sequence
  wild type local sequence
actgaagccagaccaggcgtctttccagtttattcaggggctggtccaatgctgggatatgtcatggtggcctgagaggttctcagcctc

SEQ ID NO: 196 - DNA, 89 bp, Artificial Sequence
  mutant -1
actgaagccagaccaggcgtctttccagttattcaggggctggtccaatgctgggatatgtcatggtggcctgagaggttctcagcctc

SEQ ID NO: 197 - DNA, 88 bp, Artificial Sequence
  mutant -2
actgaagccagaccaggcgtctttccagttttcaggggctggtccaatgctgggatatgtcatggtggcctgagaggttctcagcctc

SEQ ID NO: 198 - DNA, 91 bp, Artificial Sequence
  mutant +1
actgaagccagaccaggcgtctttccagttttattcaggggctggtccaatgctgggatatgtcatggtggcctgagaggttctcagcctc

SEQ ID NO: 199 - DNA, 87 bp, Artificial Sequence
  mutant -3
actgaagccagaccaggcgtctttccagtttcaggggctggtccaatgctgggatatgtcatggtggcctgagaggttctcagcctc

SEQ ID NO: 200 - DNA, 86 bp, Artificial Sequence
  mutant -4
actgaagccagaccaggcgtctttccagttcaggggctggtccaatgctgggatatgtcatggtggcctgagaggttctcagcctc

SEQ ID NO: 201 - DNA, 23 bp, Artificial Sequence
  on-target
ggaccagcccctgaataaactgg

SEQ ID NO: 202 - DNA, 23 bp, Artificial Sequence
  off1
ggaccagccacagaataaacaag

SEQ ID NO: 203 - DNA, 23 bp, Artificial Sequence
  off2
tgaccagtccatgaataaaccag

SEQ ID NO: 204 - DNA, 23 bp, Artificial Sequence
  off3
ggaccagacactgaatataccag

SEQ ID NO: 205 - DNA, 23 bp, Artificial Sequence
  off4
ggaccagccacagaataaattgg

SEQ ID NO: 206 - DNA, 23 bp, Artificial Sequence
  off5
ggatcagccacagaataaattag

SEQ ID NO: 207 - DNA, 23 bp, Artificial Sequence
  off6
ggagcatccccagaataaaccag

SEQ ID NO: 208 - DNA, 23 bp, Artificial Sequence
  off7
ggatcagcgtctgaataaacaag

SEQ ID NO: 209 - DNA, 23 bp, Artificial Sequence
  off8
agaccagccccagaacaaacaag

SEQ ID NO: 210 - DNA, 23 bp, Artificial Sequence
  off9
gtacgagcccctgaataaatagg

SEQ ID NO: 211 - DNA, 23 bp, Artificial Sequence
  off10
ggaccaaacactgaataaaccag

SEQ ID NO: 212 - DNA, 23 bp, Artificial Sequence
  off11
gcaccagccactgaattaacaag

SEQ ID NO: 213 - DNA, 23 bp, Artificial Sequence
  off12
gtaccagccactgaaaaaacagg

SEQ ID NO: 214 - DNA, 23 bp, Artificial Sequence
  off13
gaaccagcccctgattagaccag

SEQ ID NO: 215 - DNA, 23 bp, Artificial Sequence
  off14
gtaccagccactgaaaaaacagg

SEQ ID NO: 216 - DNA, 23 bp, Artificial Sequence
  off15
gtaccagcccctgcaaaaacagg

SEQ ID NO: 217 - DNA, 23 bp, Artificial Sequence
  off16
gcaccaggccttgaataaacaag

SEQ ID NO: 218 - DNA, 23 bp, Artificial Sequence
  off17
ggcccagccactgagtaaactag

SEQ ID NO: 219 - DNA, 23 bp, Artificial Sequence
  off18
ggaattgcccctgaataaacaag

SEQ ID NO: 220 - DNA, 23 bp, Artificial Sequence
  off 1
gggaacagccctgaataaacctg

SEQ ID NO: 221 - DNA, 23 bp, Artificial Sequence
  off 2
aggacgagctctgaataaccagg

SEQ ID NO: 222 - DNA, 23 bp, Artificial Sequence
  off 3
ggaacagccctgaataaacctgg

SEQ ID NO: 223 - DNA, 23 bp, Artificial Sequence
  off 4
gagttcagcccctgaataacagg

SEQ ID NO: 224 - DNA, 23 bp, Artificial Sequence
  off 5
gggaccagccccagaataaaggg

SEQ ID NO: 225 - DNA, 23 bp, Artificial Sequence
  off 6
aagccaacccctgaataaacagg

SEQ ID NO: 226 - DNA, 23 bp, Artificial Sequence
  off 7
cacacagcccctcaataaactgg

SEQ ID NO: 227 - DNA, 23 bp, Artificial Sequence
  off 8
gaggcagcccctgtataaactgg

SEQ ID NO: 228 - DNA, 23 bp, Artificial Sequence
  off 9
gaccagccccctgaataacatgg

SEQ ID NO: 229 - DNA, 23 bp, Artificial Sequence
  off 1
gtaccagcccctgacaaaacagg

SEQ ID NO: 230 - DNA, 23 bp, Artificial Sequence
  off 2
ggagcagccccggaatgaacagg

SEQ ID NO: 231 - DNA, 23 bp, Artificial Sequence
  off 3, 4, 5
ggaccagcccctgtataccctgg

SEQ ID NO: 232 - DNA, 23 bp, Artificial Sequence
  off 6
ggccctgcccctaaataaacagg

SEQ ID NO: 233 - DNA, 23 bp, Artificial Sequence
  off 7
ggatcagccccagaataacctgg

SEQ ID NO: 234 - DNA, 23 bp, Artificial Sequence
  off 8
ggactagcccctgagtacactgg